European Patent Specification EP 3 580 560 B1, published October 2, 2024. Title: METHODS FOR THE DETECTION AND TREATMENT OF LUNG CANCER. Applicant: Board of Regents, the University of Texas System. The sequence listing filed with the application follows.

SEQUENCE LISTING (4 sequences)

SEQ ID NO: 1 - protein, 702 aa, Homo sapiens
MESPSAPPHRWCIPWQRLLLTASLLTFWNPPTTAKLTIESTPFNVAEGKEVLLLVHNLPQHLFGYSWYKGERVDGNRQIIGYVIGTQQATPGPAYSGREIIYPNASLLIQNIIQNDTGFYTLHVIKSDLVNEEATGQFRVYPELPKPSISSNNSKPVEDKDAVAFTCEPETQDATYLWWVNNQSLPVSPRLQLSNGNRTLTLFNVTRNDTASYKCETQNPVSARRSDSVILNVLYGPDAPTISPLNTSYRSGENLNLSCHAASNPPAQYSWFVNGTFQQSTQELFIPNITVNNSGSYTCQAHNSDTGLNRTTVTTITVYAEPPKPFITSNNSNPVEDEDAVALTCEPEIQNTTYLWWVNNQSLPVSPRLQLSNDNRTLTLLSVTRNDVGPYECGIQNKLSVDHSDPVILNVLYGPDDPTISPSYTYYRPGVNLSLSCHAASNPPAQYSWLIDGNIQQHTQELFISNITEKNSGLYTCQANNSASGHSRTTVKTITVSAELPKPSISSNNSKPVEDKDAVAFTCEPEAQNTTYLWWVNGQSLPVSPRLQLSNGNRTLTLFNVTRNDARAYVCGIQNSVSANRSDPVTLDVLYGPDTPIISPPDSSYLSGANLNLSCHSASNPSPQYSWRINGIPQQHTQVLFIAKITPNNNGTYACFVSNLATGRNNSIVKSITVSASGTSPGLSAGATVGIMIGVLVGVALI

SEQ ID NO: 2 - protein, 14451 aa, Homo sapiens
MLKPSGLPGSSSPTRSLMTGSRSTKATPEMDSGLTGATLSPKTSTGAIVVTEHTLPFTSPDKTLASPTSSVVGRTTQSLGVMSSALPESTSRGMTHSEQRTSPSLSPQVNGTPSRNYPATSMVSGLSSPRTRTSSTEGNFTKEASTYTLTVETTSGPVTEKYTVPTETSTTEGDSTETPWDTRYIPVKITSPMKTFADSTASKENAPVSMTPAETTVTDSHTPGRTNPSFGTLYSSFLDLSPKGTPNSRGETSLELILSTTGYPFSSPEPGSAGHSRISTSAPLSSSASVLDNKISETSIFSGQSLTSPLSPGVPEARASTMPNSAIPFSMTLSNAETSAERVRSTISSLGTPSISTKQTAETILTFHAFAETMDIPSTHIAKTLASEWLGSPGTLGGTSTSALTTTSPSTTLVSEETNTHHSTSGKETEGTLNTSMTPLETSAPGEESEMTATLVPTLGFTTLDSKIRSPSQVSSSHPTRELRTTGSTSGRQSSSTAAHGSSDILRATTSSTSKASSWTSESTAQQFSEPQHTQWVETSPSMKTERPPASTSVAAPITTSVPSVVSGFTTLKTSSTKGIWLEETSADTLIGESTAGPTTHQFAVPTGISMTGGSSTRGSQGTTHLLTRATASSETSADLTLATNGVPVSVSPAVSKTAAGSSPPGGTKPSYTMVSSVIPETSSLQSSAFREGTSLGLTPLNTRHPFSSPEPDSAGHTKISTSIPLLSSASVLEDKVSATSTFSHHKATSSITTGTPEISTKTKPSSAVLSSMTLSNAATSPERVRNATSPLTHPSPSGEETAGSVLTLSTSAETTDSPNIHPTGTLTSESSESPSTLSLPSVSGVKTTFSSSTPSTHLFTSGEETEETSNPSVSQPETSVSRVRTTLASTSVPTPVFPTMDTWPTRSAQFSSSHLVSELRATSSTSVTNSTGSALPKISHLTGTATMSQTNRDTFNDSAAPQSTTWPETSPRFKTGLPSATTTVSTSATSLSATVMVSKFTSPATSSMEATSIREPSTTILTTETTNGPGSMAVASTNIPIGKGYITEGRLDTSHLPIGTTASSETSMDFTMAKESVSMSVSPSQSMDAAGSSTPGRTSQFVDTFSDDVYHLTSREITIPRDGTSSALTPQMTATHPPSPDPGSARSTWLGILSSSPSSPTPKVTMSSTFSTQRVTTSMIMDTVETSRWNMPNLPSTTSLTPSNIPTSGAIGKSTLVPLDTPSPATSLEASEGGLPTLSTYPESTNTPSIHLGAHASSESPSTIKLTMASVVKPGSYTPLTFPSIETHIHVSTARMAYSSGSSPEMTAPGETNTGSTWDPTTYITTTDPKDTSSAQVSTPHSVRTLRTTENHPKTESATPAAYSGSPKISSSPNLTSPATKAWTITDTTEHSTQLHYTKLAEKSSGFETQSAPGPVSVVIPTSPTIGSSTLELTSDVPGEPLVLAPSEQTTITLPMATWLSTSLTEEMASTDLDISSPSSPMSTFAIFPPMSTPSHELSKSEADTSAIRNTDSTTLDQHLGIRSLGRTGDLTTVPITPLTTTWTSVIEHSTQAQDTLSATMSPTHVTQSLKDQTSIPASASPSHLTEVYPELGTQGRSSSEATTFWKPSTDTLSREIETGPTNIQSTPPMDNTTTGSSSSGVTLGIAHLPIGTSSPAETSTNMALERRSSTATVSMAGTMGLLVTSAPGRSISQSLGRVSSVLSESTTEGVTDSSKGSSPRLNTQGNTALSSSLEPSYAEGSQMSTSIPLTSSPTTPDVEFIGGSTFWTKEVTTVMTSDISKSSARTESSSATLMSTALGSTENTGKEKLRTASMDLPSPTPSMEVTPWISLTLSNAPNTTDSLDLSHGVHTSSAGTLATDRSLNTGVTRASRLENGSDTSSKSLSMGNSTHTSMTYTEKSEVSSSIHPRPETSAPGAETTLTSTPGNRAISLTLPFSSIPVEEVISTGITSGPDINSAPMTHSPITPPTIVWTSTGTIEQSTQPLHAVSSEKVSVQTQSTPYVNSVAVSASPTHENSVSSGSSTSSPYSSASLESLDSTISRRNAITSWLWDLTTSLPTTTWPSTSLSEALSSGHSGVSNPSSTTTEFPLFSAASTSAAKQRNPETETHGPQNTAASTLNTDASSVTGLSETPVGASISSEVPLPMAITSRSDVSGLTSESTANPSLGTASSAGTKLTRTISLPTSESLVSFRMNKDPWTVSIPLGSHPTTNTETSIPVNSAGPPGLSTVASDVIDTPSDGAESIPTVSFSPSPDTEVTTISHFPEKTTHSFRTISSLTHELTSRVTPIPGDWMSSAMSTKPTGASPSITLGERRTITSAAPTTSPIVLTASFTETSTVSLDNETTVKTSDILDARKTNELPSDSSSSSDLINTSIASSTMDVTKTASISPTSISGMTASSSPSLFSSDRPQVPTSTTETNTATSPSVSSNTYSLDGGSNVGGTPSTLPPFTITHPVETSSALLAWSRPVRTFSTMVSTDTASGENPTSSNSVVTSVPAPGTWTSVGSTTDLPAMGFLKTSPAGEAHSLLASTIEPATAFTPHLSAAVVTGSSATSEASLLTTSESKAIHSSPQTPTTPTSGANWETSATPESLLVVTETSDTTLTSKILVTDTILFSTVSTPPSKFPSTGTLSGASFPTLLPDTPAIPLTATEPTSSLATSFDSTPLVTIASDSLGTVPETTLTMSETSNGDALVLKTVSNPDRSIPGITIQGVTESPLHPSSTSPSKIVAPRNTTYEGSITVALSTLPAGTTGSLVFSQSSENSETTALVDSSAGLERASVMPLTTGSQGMASSGGIRSGSTHSTGTKTFSSLPLTMNPGEVTAMSEITTNRLTATQSTAPKGIPVKPTSAESGLLTPVSASSSPSKAFASLTTAPPTWGIPQSTLTFEFSEVPSLDTKSASLPTPGQSLNTIPDSDASTASSSLSKSPEKNPRARMMTSTKAISASSFQSTGFTETPEGSASPSMAGHEPRVPTSGTGDPRYASESMSYPDPSKASSAMTSTSLASKLTTLFSTGQAARSGSSSSPISLSTEKETSFLSPTASTSRKTSLFLGPSMARQPNILVHLQTSALTLSPTSTLNMSQEEPPELTSSQTIAEEEGTTAETQTLTFTPSETPTSLLPVSSPTEPTARRKSSPETWASSISVPAKTSLVETTDGTLVTTIKMSSQAAQGNSTWPAPAEETGSSPAGTSPGSPEMSTTLKIMSSKEPSISPEIRSTVRNSPWKTPETTVPMETTVEPVTLQSTALGSGSTSISHLPTGTTSPTKSPTENMLATERVSLSPSPPEAWTNLYSGTPGGTRQSLATMSSVSLESPTARSITGTGQQSSPELVSKTTGMEFSMWHGSTGGTTGDTHVSLSTSSNILEDPVTSPNSVSSLTDKSKHKTETWVSTTAIPSTVLNNKIMAAEQQTSRSVDEAYSSTSSWSDQTSGSDITLGASPDVTNTLYITSTAQTTSLVSLPSGDQGITSLTNPSGGKTSSASSVTSPSIGLETLRANVSAVKSDIAPTAGHLSQTSSPAEVSILDVTTAPTPGISTTITTMGTNSISTTTPNPEVGMSTMDSTPATERRTTSTEHPSTWSSTAASDSWTVTDMTSNLKVARSPGTISTMHTTSFLASSTELDSMSTPHGRITVIGTSLVTPSSDASAVKTETSTSERTLSPSDTTASTPISTFSRVQRMSISVPDILSTSWTPSSTEAEDVPVSMVSTDHASTKTDPNTPLSTFLFDSLSTLDWDTGRSLSSATATTSAPQGATTPQELTLETMISPATSQLPFSIGHITSAVTPAAMARSSGVTFSRPDPTSKKAEQTSTQLPTTTSAHPGQVPRSAATTLDVIPHTAKTPDATFQRQGQTALTTEARATSDSWNEKEKSTPSAPWITEMMNSVSEDTIKEVTSSSSVLRTLNTLDINLESGTTSSPSWKSSPYERIAPSESTTDKEAIHPSTNTVETTGWVTSSEHASHSTIPAHSASSKLTSPVVTTSTREQAIVSMSTTTWPESTRARTEPNSFLTIELRDVSPYMDTSSTTQTSIISSPGSTAITKGPRTEITSSKRISSSFLAQSMRSSDSPSEAITRLSNFPAMTESGGMILAMQTSPPGATSLSAPTLDTSATASWTGTPLATTQRFTYSEKTTLFSKGPEDTSQPSPPSVEETSSSSSLVPIHATTSPSNILLTSQGHSPSSTPPVTSVFLSETSGLGKTTDMSRISLEPGTSLPPNLSSTAGEALSTYEASRDTKAIHHSADTAVTNMEATSSEYSPIPGHTKPSKATSPLVTSHIMGDITSSTSVFGSSETTEIETVSSVNQGLQERSTSQVASSATETSTVITHVSSGDATTHVTKTQATFSSGTSISSPHQFITSTNTFTDVSTNPSTSLIMTESSGVTITTQTGPTGAATQGPYLLDTSTMPYLTETPLAVTPDFMQSEKTTLISKGPKDVSWTSPPSVAETSYPSSLTPFLVTTIPPATSTLQGQHTSSPVSATSVLTSGLVKTTDMLNTSMEPVTNSPQNLNNPSNEILATLAATTDIETIHPSINKAVTNMGTASSAHVLHSTLPVSSEPSTATSPMVPASSMGDALASISIPGSETTDIEGEPTSSLTAGRKENSTLQEMNSTTESNIILSNVSVGAITEATKMEVPSFDATFIPTPAQSTKFPDIFSVASSRLSNSPPMTISTHMTTTQTGSSGATSKIPLALDTSTLETSAGTPSVVTEGFAHSKITTAMNNDVKDVSQTNPPFQDEASSPSSQAPVLVTTLPSSVAFTPQWHSTSSPVSMSSVLTSSLVKTAGKVDTSLETVTSSPQSMSNTLDDISVTSAATTDIETTHPSINTVVTNVGTTGSAFESHSTVSAYPEPSKVTSPNVTTSTMEDTTISRSIPKSSKTTRTETETTSSLTPKLRETSISQEITSSTETSTVPYKELTGATTEVSRTDVTSSSSTSFPGPDQSTVSLDISTETNTRLSTSPIMTESAEITITTQTGPHGATSQDTFTMDPSNTTPQAGIHSAMTHGFSQLDVTTLMSRIPQDVSWTSPPSVDKTSSPSSFLSSPAMTTPSLISSTLPEDKLSSPMTSLLTSGLVKITDILRTRLEPVTSSLPNFSSTSDKILATSKDSKDTKEIFPSINTEETNVKANNSGHESHSPALADSETPKATTQMVITTTVGDPAPSTSMPVHGSSETTNIKREPTYFLTPRLRETSTSQESSFPTDTSFLLSKVPTGTITEVSSTGVNSSSKISTPDHDKSTVPPDTFTGEIPRVFTSSIKTKSAEMTITTQASPPESASHSTLPLDTSTTLSQGGTHSTVTQGFPYSEVTTLMGMGPGNVSWMTTPPVEETSSVSSLMSSPAMTSPSPVSSTSPQSIPSSPLPVTALPTSVLVTTTDVLGTTSPESVTSSPPNLSSITHERPATYKDTAHTEAAMHHSTNTAVTNVGTSGSGHKSQSSVLADSETSKATPLMSTTSTLGDTSVSTSTPNISQTNQIQTEPTASLSPRLRESSTSEKTSSTTETNTAFSYVPTGAITQASRTEISSSRTSISDLDRPTIAPDISTGMITRLFTSPIMTKSAEMTVTTQTTTPGATSQGILPWDTSTTLFQGGTHSTVSQGFPHSEITTLRSRTPGDVSWMTTPPVEETSSGFSLMSPSMTSPSPVSSTSPESIPSSPLPVTALLTSVLVTTTNVLGTTSPEPVTSSPPNLSSPTQERLTTYKDTAHTEAMHASMHTNTAVANVGTSISGHESQSSVPADSHTSKATSPMGITFAMGDTSVSTSTPAFFETRIQTESTSSLIPGLRDTRTSEEINTVTETSTVLSEVPTTTTTEVSRTEVITSSRTTISGPDHSKMSPYISTETITRLSTFPFVTGSTEMAITNQTGPIGTISQATLTLDTSSTASWEGTHSPVTQRFPHSEETTTMSRSTKGVSWQSPPSVEETSSPSSPVPLPAITSHSSLYSAVSGSSPTSALPVTSLLTSGRRKTIDMLDTHSELVTSSLPSASSFSGEILTSEASTNTETIHFSENTAETNMGTTNSMHKLHSSVSIHSQPSGHTPPKVTGSMMEDAIVSTSTPGSPETKNVDRDSTSPLTPELKEDSTALVMNSTTESNTVFSSVSLDAATEVSRAEVTYYDPTFMPASAQSTKSPDISPEASSSHSNSPPLTISTHKTIATQTGPSGVTSLGQLTLDTSTIATSAGTPSARTQDFVDSETTSVMNNDLNDVLKTSPFSAEEANSLSSQAPLLVTTSPSPVTSTLQEHSTSSLVSVTSVPTPTLAKITDMDTNLEPVTRSPQNLRNTLATSEATTDTHTMHPSINTAVANVGTTSSPNEFYFTVSPDSDPYKATSAVVITSTSGDSIVSTSMPRSSAMKKIESETTFSLIFRLRETSTSQKIGSSSDTSTVFDKAFTAATTEVSRTELTSSSRTSIQGTEKPTMSPDTSTRSVTMLSTFAGLTKSEERTIATQTGPHRATSQGTLTWDTSITTSQAGTHSAMTHGFSQLDLSTLTSRVPEYISGTSPPSVEKTSSSSSLLSLPAITSPSPVPTTLPESRPSSPVHLTSLPTSGLVKTTDMLASVASLPPNLGSTSHKIPTTSEDIKDTEKMYPSTNIAVTNVGTTTSEKESYSSVPAYSEPPKVTSPMVTSFNIRDTIVSTSMPGSSEITRIEMESTFSLAHGLKGTSTSQDPIVSTEKSAVLHKLTTGATETSRTEVASSRRTSIPGPDHSTESPDISTEVIPSLPISLGITESSNMTIITRTGPPLGSTSQGTFTLDTPTTSSRAGTHSMATQEFPHSEMTTVMNKDPEILSWTIPPSIEKTSFSSSLMPSPAMTSPPVSSTLPKTIHTTPSPMTSLLTPSLVMTTDTLGTSPEPTTSSPPNLSSTSHEILTTDEDTTAIEAMHPSTSTAATNVETTSSGHGSQSSVLADSEKTKATAPMDTTSTMGHTTVSTSMSVSSETTKIKRESTYSLTPGLRETSISQNASFSTDTSIVLSEVPTGTTAEVSRTEVTSSGRTSIPGPSQSTVLPEISTRTMTRLFASPTMTESAEMTIPTQTGPSGSTSQDTLTLDTSTTKSQAKTHSTLTQRFPHSEMTTLMSRGPGDMSWQSSPSLENPSSLPSLLSLPATTSPPPISSTLPVTISSSPLPVTSLLTSSPVTTTDMLHTSPELVTSSPPKLSHTSDERLTTGKDTTNTEAVHPSTNTAASNVEIPSSGHESPSSALADSETSKATSPMFITSTQEDTTVAISTPHFLETSRIQKESISSLSPKLRETGSSVETSSAIETSAVLSEVSIGATTEISRTEVTSSSRTSISGSAESTMLPEISTTRKIIKFPTSPILAESSEMTIKTQTSPPGSTSESTFTLDTSTTPSLVITHSTMTQRLPHSEITTLVSRGAGDVPRPSSLPVEETSPPSSQLSLSAMISPSPVSSTLPASSHSSSASVTSLLTPGQVKTTEVLDASAEPETSSPPSLSSTSVEILATSEVTTDTEKIHPFSNTAVTKVGTSSSGHESPSSVLPDSETTKATSAMGTISIMGDTSVSTLTPALSNTRKIQSEPASSLTTRLRETSTSEETSLATEANTVLSKVSTGATTEVSRTEAISFSRTSMSGPEQSTMSQDISIGTIPRISASSVLTESAKMTITTQTGPSESTLESTLNLNTATTPSWVETHSIVIQGFPHPEMTTSMGRGPGGVSWPSPPFVKETSPPSSPLSLPAVTSPHPVSTTFLAHIPPSPLPVTSLLTSGPATTTDILGTSTEPGTSSSSSLSTTSHERLTTYKDTAHTEAVHPSTNTGGTNVATTSSGYKSQSSVLADSSPMCTTSTMGDTSVLTSTPAFLETRRIQTELASSLTPGLRESSGSEGTSSGTKMSTVLSKVPTGATTEISKEDVTSIPGPAQSTISPDISTRTVSWFSTSPVMTESAEITMNTHTSPLGATTQGTSTLDTSSTTSLTMTHSTISQGFSHSQMSTLMRRGPEDVSWMSPPLLEKTRPSFSLMSSPATTSPSPVSSTLPESISSSPLPVTSLLTSGLAKTTDMLHKSSEPVTNSPANLSSTSVEILATSEVTTDTEKTHPSSNRTVTDVGTSSSGHESTSFVLADSQTSKVTSPMVITSTMEDTSVSTSTPGFFETSRIQTEPTSSLTLGLRKTSSSEGTSLATEMSTVLSGVPTGATAEVSRTEVTSSSRTSISGFAQLTVSPETSTETITRLPTSSIMTESAEMMIKTQTDPPGSTPESTHTVDISTTPNWVETHSTVTQRFSHSEMTTLVSRSPGDMLWPSQSSVEETSSASSLLSLPATTSPSPVSSTLVEDFPSASLPVTSLLNPGLVITTDRMGISREPGTSSTSNLSSTSHERLTTLEDTVDTEDMQPSTHTAVTNVRTSISGHESQSSVLSDSETPKATSPMGTTYTMGETSVSISTSDFFETSRIQIEPTSSLTSGLRETSSSERISSATEGSTVLSEVPSGATTEVSRTEVISSRGTSMSGPDQFTISPDISTEAITRLSTSPIMTESAESAITIETGSPGATSEGTLTLDTSTTTFWSGTHSTASPGFSHSEMTTLMSRTPGDVPWPSLPSVEEASSVSSSLSSPAMTSTSFFSTLPESISSSPHPVTALLTLGPVKTTDMLRTSSEPETSSPPNLSSTSAEILATSEVTKDREKIHPSSNTPVVNVGTVIYKHLSPSSVLADLVTTKPTSPMATTSTLGNTSVSTSTPAFPETMMTQPTSSLTSGLREISTSQETSSATERSASLSGMPTGATTKVSRTEALSLGRTSTPGPAQSTISPEISTETITRISTPLTTTGSAEMTITPKTGHSGASSQGTFTLDTSSRASWPGTHSAATHRSPHSGMTTPMSRGPEDVSWPSRPSVEKTSPPSSLVSLSAVTSPSPLYSTPSESSHSSPLRVTSLFTPVMMKTTDMLDTSLEPVTTSPPSMNITSDESLATSKATMETEAIQLSENTAVTQMGTISARQEFYSSYPGLPEPSKVTSPVVTSSTIKDIVSTTIPASSEITRIEMESTSTLTPTPRETSTSQEIHSATKPSTVPYKALTSATIEDSMTQVMSSSRGPSPDQSTMSQDISTEVITRLSTSPIKTESTEMTITTQTGSPGATSRGTLTLDTSTTFMSGTHSTASQGFSHSQMTALMSRTPGDVPWLSHPSVEEASSASFSLSSPVMTSSSPVSSTLPDSIHSSSLPVTSLLTSGLVKTTELLGTSSEPETSSPPNLSSTSAEILAITEVTTDTEKLEMTNVVTSGYTHESPSSVLADSVTTKATSSMGITYPTGDTNVLTSTPAFSDTSRIQTKSKLSLTPGLMETSISEETSSATEKSTVLSSVPTGATTEVSRTEAISSSRTSIPGPAQSTMSSDTSMETITRISTPLTRKESTDMAITPKTGPSGATSQGTFTLDSSSTASWPGTHSATTQRFPQSVVTTPMSRGPEDVSWPSPLSVEKNSPPSSLVSSSSVTSPSPLYSTPSGSSHSSPVPVTSLFTSIMMKATDMLDASLEPETTSAPNMNITSDESLAASKATTETEAIHVFENTAASHVETTSATEELYSSSPGFSEPTKVISPVVTSSSIRDNMVSTTMPGSSGITRIEIESMSSLTPGLRETRTSQDITSSTETSTVLYKMPSGATPEVSRTEVMPSSRTSIPGPAQSTMSLDISDEVVTRLSTSPIMTESAEITITTQTGYSLATSQVTLPLGTSMTFLSGTHSTMSQGLSHSEMTNLMSRGPESLSWTSPRFVETTRSSSSLTSLPLTTSLSPVSSTLLDSSPSSPLPVTSLILPGLVKTTEVLDTSSEPKTSSSPNLSSTSVEIPATSEIMTDTEKIHPSSNTAVAKVRTSSSVHESHSSVLADSETTITIPSMGITSAVDDTTVFTSNPAFSETRRIPTEPTFSLTPGFRETSTSEETTSITETSAVLYGVPTSATTEVSMTEIMSSNRIHIPDSDQSTMSPDIITEVITRLSSSSMMSESTQMTITTQKSSPGATAQSTLTLATTTAPLARTHSTVPPRFLHSEMTTLMSRSPENPSWKSSLFVEKTSSSSSLLSLPVTTSPSVSSTLPQSIPSSSFSVTSLLTPGMVKTTDTSTEPGTSLSPNLSGTSVEILAASEVTTDTEKIHPSSSMAVTNVGTTSSGHELYSSVSIHSEPSKATYPVGTPSSMAETSISTSMPANFETTGFEAEPFSHLTSGFRKTNMSLDTSSVTPTNTPSSPGSTHLLQSSKTDFTSSAKTSSPDWPPASQYTEIPVDIITPFNASPSITESTGITSFPESRFTMSVTESTHHLSTDLLPSAETISTGTVMPSLSEAMTSFATTGVPRAISGSGSPFSRTESGPGDATLSTIAESLPSSTPVPFSSSTFTTTDSSTIPALHEITSSSATPYRVDTSLGTESSTTEGRLVMVSTLDTSSQPGRTSSSPILDTRMTESVELGTVTSAYQVPSLSTRLTRTDGIMEHITKIPNEAAHRGTIRPVKGPQTSTSPASPKGLHTGGTKRMETTTTALKTTTTALKTTSRATLTTSVYTPTLGTLTPLNASMQMASTIPTEMMITTPYVFPDVPETTSSLATSLGAETSTALPRTTPSVFNRESETTASLVSRSGAERSPVIQTLDVSSSEPDTTASWVIHPAETIPTVSKTTPNFFHSELDTVSSTATSHGADVSSAIPTNISPSELDALTPLVTISGTDTSTTFPTLTKSPHETETRTTWLTHPAETSSTIPRTIPNFSHHESDATPSIATSPGAETSSAIPIMTVSPGAEDLVTSQVTSSGTDRNMTIPTLTLSPGEPKTIASLVTHPEAQTSSAIPTSTISPAVSRLVTSMVTSLAAKTSTTNRALTNSPGEPATTVSLVTHPAQTSPTVPWTTSIFFHSKSDTTPSMTTSHGAESSSAVPTPTVSTEVPGVVTPLVTSSRAVISTTIPILTLSPGEPETTPSMATSHGEEASSAIPTPTVSPGVPGVVTSLVTSSRAVTSTTIPILTFSLGEPETTPSMATSHGTEAGSAVPTVLPEVPGMVTSLVASSRAVTSTTLPTLTLSPGEPETTPSMATSHGAEASSTVPTVSPEVPGVVTSLVTSSSGVNSTSIPTLILSPGELETTPSMATSHGAEASSAVPTPTVSPGVSGVVTPLVTSSRAVTSTTIPILTLSSSEPETTPSMATSHGVEASSAVLTVSPEVPGMVTSLVTSSRAVTSTTIPTLTISSDEPETTTSLVTHSEAKMISAIPTLAVSPTVQGLVTSLVTSSGSETSAFSNLTVASSQPETIDSWVAHPGTEASSVVPTLTVSTGEPFTNISLVTHPAESSSTLPRTTSRFSHSELDTMPSTVTSPEAESSSAISTTISPGIPGVLTSLVTSSGRDISATFPTVPESPHESEATASWVTHPAVTSTTVPRTTPNYSHSEPDTTPSIATSPGAEATSDFPTITVSPDVPDMVTSQVTSSGTDTSITIPTLTLSSGEPETTTSFITYSETHTSSAIPTLPVSPGASKMLTSLVISSGTDSTTTFPTLTETPYEPETTAIQLIHPAETNTMVPRTTPKFSHSKSDTTLPVAITSPGPEASSAVSTTTISPDMSDLVTSLVPSSGTDTSTTFPTLSETPYEPETTATWLTHPAETSTTVSGTIPNFSHRGSDTAPSMVTSPGVDTRSGVPTTTIPPSIPGVVTSQVTSSATDTSTAIPTLTPSPGEPETTASSATHPGTQTGFTVPIRTVPSSEPDTMASWVTHPPQTSTPVSRTTSSFSHSSPDATPVMATSPRTEASSAVLTTISPGAPEMVTSQITSSGAATSTTVPTLTHSPGMPETTALLSTHPRTETSKTFPASTVFPQVSETTASLTIRPGAETSTALPTQTTSSLFTLLVTGTSRVDLSPTASPGVSAKTAPLSTHPGTETSTMIPTSTLSLGLLETTGLLATSSSAETSTSTLTLTVSPAVSGLSSASITTDKPQTVTSWNTETSPSVTSVGPPEFSRTVTGTTMTLIPSEMPTPPKTSHGEGVSPTTILRTTMVEATNLATTGSSPTVAKTTTTFNTLAGSLFTPLTTPGMSTLASESVTSRTSYNHRSWISTTSSYNRRYWTPATSTPVTSTFSPGISTSSIPSSTAATVPFMVPFTLNFTITNLQYEEDMRHPGSRKFNATERELQGLLKPLFRNSSLEYLYSGCRLASLRPEKDSSATAVDAICTHRPDPEDLGLDRERLYWELSNLTNGIQELGPYTLDRNSLYVNGFTHRSSMPTTSTPGTSTVDVGTSGTPSSSPSPTTAGPLLMPFTLNFTITNLQYEEDMRRTGSRKFNTMESVLQGLLKPLFKNTSVGPLYSGCRLTLLRPEKDGAATGVDAICTHRLDPKSPGLNREQLYWELSKLTNDIEELGPYTLDRNSLYVNGFTHQSSVSTTSTPGTSTVDLRTSGTPSSLSSPTIMAAGPLLVPFTLNFTITNLQYGEDMGHPGSRKFNTTERVLQGLLGPIFKNTSVGPLYSGCRLTSLRSEKDGAATGVDAICIHHLDPKSPGLNRERLYWELSQLTNGIKELGPYTLDRNSLYVNGFTHRTSVPTSSTPGTSTVDLGTSGTPFSLPSPATAGPLLVLFTLNFTITNLKYEEDMHRPGSRKFNTTERVLQTLLGPMFKNTSVGLLYSGCRLTLLRSEKDGAATGVDAICTHRLDPKSPGVDREQLYWELSQLTNGIKELGPYTLDRNSLYVNGFTHWIPVPTSSTPGTSTVDLGSGTPSSLPSPTTAGPLLVPFTLNFTITNLKYEEDMHCPGSRKFNTTERVLQSLLGPMFKNTSVGPLYSGCRLTLLRSEKDGAATGVDAICTHRLDPKSPGVDREQLYWELSQLTNGIKELGPYTLDRNSLYVNGFTHQTSAPNTSTPGTSTVDLGTSGTPSSLPSPTSAGPLLVPFTLNFTITNLQYEEDMHHPGSRKFNTTERVLQGLLGPMFKNTSVGLLYSGCRLTLLRPEKNGAATGMDAICSHRLDPKSPGLNREQLYWELSQLTHGIKELGPYTLDRNSLYVNGFTHRSSVAPTSTPGTSTVDLGTSGTPSSLPSPTTAVPLLVPFTLNFTITNLQYGEDMRHPGSRKFNTTERVLQGLLGPLFKNSSVGPLYSGCRLISLRSEKDGAATGVDAICTHHLNPQSPGLDREQLYWQLSQMTNGIKELGPYTLDRNSLYVNGFTHRSSGLTTSTPWTSTVDLGTSGTPSPVPSPTTTGPLLVPFTLNFTITNLQYEENMGHPGSRKFNITESVLQGLLKPLFKSTSVGPLYSGCRLTLLRPEKDGVATRVDAICTHRPDPKIPGLDRQQLYWELSQLTHSITELGPYTLDRDSLYVNGFTQRSSVPTTSTPGTFTVQPETSETPSSLPGPTATGPVLLPFTLNFTITNLQYEEDMRRPGSRKFNTTERVLQGLLMPLFKNTSVSSLYSGCRLTLLRPEKDGAATRVDAVCTHRPDPKSPGLDRERLYWKLSQLTHGITELGPYTLDRHSLYVNGFTHQSSMTTTRTPDTSTMHLATSRTPASLSGPMTASPLLVLFTINFTITNLRYEENMHHPGSRKFNTTERVLQGLLRPVFKNTSVGPLYSGCRLTLLRPKKDGAATKVDAICTYRPDPKSPGLDREQLYWELSQLTHSITELGPYTLDRDSLYVNGFTQRSSVPTTSIPGTPTVDLGTSGTPVSKPGPSAASPLLVLFTLNFTITNLRYEENMQHPGSRKFNTTERVLQGLLRSLFKSTSVGPLYSGCRLTLLRPEKDGTATGVDAICTHHPDPKSPRLDREQLYWELSQLTHNITELGPYALDNDSLFVNGFTHRSSVSTTSTPGTPTVYLGASKTPASIFGPSAASHLLILFTLNFTITNLRYEENMWPGSRKFNTTERVLQGLLRPLFKNTSVGPLYSGCRLTLLRPEKDGEATGVDAICTHRPDPTGPGLDREQLYLELSQLTHSITELGPYTLDRDSLYVNGFTHRSSVPTTSTGVVSEEPFTLNFTINNLRYMADMGQPGSLKFNITDNVMQHLLSPLFQRSSLGARYTGCRVIALRSVKNGAETRVDLLCTYLQPLSGPGLPIKQVFHELSQQTHGITRLGPYSLDKDSLYLNGYNEPGPDEPPTTPKPATTFLPPLSEATTAMGYHLKTLTLNFTISNLQYSPDMGKGSATFNSTEGVLQHLLRPLFQKSSMGPFYLGCQLISLRPEKDGAATGVDTTCTYHPDPVGPGLDIQQLYWELSQLTHGVTQLGFYVLDRDSLFINGYAPQNLSIRGEYQINFHIVNWNLSNPDPTSSEYITLLRDIQDKVTTLYKGSQLHDTFRFCLVTNLTMDSVLVTVKALFSSNLDPSLVEQVFLDKTLNASFHWLGSTYQLVDIHVTEMESSVYQPTSSSSTQHFYLNFTITNLPYSQDKAQPGTTNYQRNKRNIEDALNQLFRNSSIKSYFSDCQVSTFRSVPNRHHTGVDSLCNFSPLARRVDRVAIYEEFLRMTRNGTQLQNFTLDRSSVLVDGYSPNRNEPLTGNSDLP

SEQ ID NO: 3 - protein, 400 aa, Homo sapiens
MTSYSYRQSSATSSFGGLGGGSVRFGPGVAFRAPSIHGGSGGRGVSVSSARFVSSSSSGAYGGGYGGVLTASDGLLAGNEKLTMQNLNDRLASYLDKVRALEAANGELEVKIRDWYQKQGPGPSRDYSHYYTTIQDLRDKILGATIENSRIVLQIDNARLAADDFRTKFETEQALRMSVEADINGLRRVLDELTLARTDLEMQIEGLKEELAYLKKNHEEEISTLRGQVGGQVSVEVDSAPGTDLAKILSDMRSQYEVMAEQNRKDAEAWFTSRTEELNREVAGHTEQLQMSRSEVTDLRRTLQGLEIELQSQLSMKAALEDTLAETEARFGAQLAHIQALISGIEAQLGDVRADSERQNQEYQRLMDIKSRLEQEIATYRSLLEGQEDHYNNLSASKVL

SEQ ID NO: 4 - protein, 381 aa, Homo sapiens
MAESHLLQWLLLLLPTLCGPGTAAWTTSSLACAQGPEFWCQSLEQALQCRALGHCLQEVWGHVGADDLCQECEDIVHILNKMAKEAIFQDTMRKFLEQECNVLPLKLLMPQCNQVLDDYFPLVIDYFQNQTDSNGICMHLGLCKSRQPEPEQEPGMSDPLPKPLRDPLPDPLLDKLVLPVLPGALQARPGPHTQDLSEQQFPIPLPYCWLCRALIKRIQAMIPKGALAVAVAQVCRVVPLVAGGICQCLAERYSVILLDTLLGRMLPQLVCRLVLRCSMDDSAGPRSPTGEWLPRDSECHLCMSVTTQAGNSSEQAIPQAMLQACVGSWLDREKCKQFVEQHTPQLLTLVPRGWDAHTTCQALGVCGTMSSPLQCIHSPDL